European Patent Application EP 4 545 650 A1, published April 30, 2025. Title: ADDITIVE FOR PCR AMPLIFICATION, MULTIPLEX PCR AMPLIFICATION KIT, AND USE THEREOF. Applicant: GeneMind Biosciences Co., Ltd. Application EP. The sequence listing filed with the application follows.

SEQUENCE LISTING (176 sequences)

SEQ ID NO: 1 - DNA, 21 bp, synthetic construct
  source 1..21: mol_type = other DNA
ggaaactgttgtcccatttcg

SEQ ID NO: 2 - DNA, 20 bp, synthetic construct
  source 1..20: mol_type = other DNA
cacgttacgctcgtggacat

SEQ ID NO: 3 - DNA, 20 bp, synthetic construct
  source 1..20: mol_type = other DNA
ccgcgatcaaggagttcttc

SEQ ID NO: 4 - DNA, 18 bp, synthetic construct
  source 1..18: mol_type = other DNA
gggcggggctcaattgcc

SEQ ID NO: 5 - DNA, 20 bp, synthetic construct
  source 1..20: mol_type = other DNA
cagctacatcgactatgcga

SEQ ID NO: 6 - DNA, 18 bp, synthetic construct
  source 1..18: mol_type = other DNA
ctgcggtgaatacgttcc

SEQ ID NO: 7 - DNA, 18 bp, synthetic construct
  source 1..18: mol_type = other DNA
ccatcggcgccggtatcg

SEQ ID NO: 8 - DNA, 21 bp, synthetic construct
  source 1..21: mol_type = other DNA
tgcgtggtctgggcgccaccg

SEQ ID NO: 9 - DNA, 20 bp, synthetic construct
  source 1..20: mol_type = other DNA
ccaaccatccagcagctggt

SEQ ID NO: 10 - DNA, 22 bp, synthetic construct
  source 1..22: mol_type = other DNA
aagttggttccgttcggtgcat

SEQ ID NO: 11 - DNA, 19 bp, synthetic construct
  source 1..19: mol_type = other DNA
ggatgcctgtccaccaggt

SEQ ID NO: 12 - DNA, 20 bp, synthetic construct
  source 1..20: mol_type = other DNA
cctgcgagcgtaggcgtcgg

SEQ ID NO: 13 - DNA, 18 bp, synthetic construct
  source 1..18: mol_type = other DNA
ggttttgggtctgacgac

SEQ ID NO: 14 - DNA, 20 bp, synthetic construct
  source 1..20: mol_type = other DNA
gggctggaagagctcgtatg

SEQ ID NO: 15 - DNA, 21 bp, synthetic construct
  source 1..21: mol_type = other DNA
caggactgaacgggatacgaa

SEQ ID NO: 16 - DNA, 20 bp, synthetic construct
  source 1..20: mol_type = other DNA
acacgatctcgtcgctaacc

SEQ ID NO: 17 - DNA, 21 bp, synthetic construct
  source 1..21: mol_type = other DNA
gcgcatccacagactggcgtc

SEQ ID NO: 18 - DNA, 19 bp, synthetic construct
  source 1..19: mol_type = other DNA
gggcttcggtgtacctcat

SEQ ID NO: 19 - DNA, 19 bp, synthetic construct
  source 1..19: mol_type = other DNA
ctcgcccactacagacaag

SEQ ID NO: 20 - DNA, 20 bp, synthetic construct
  source 1..20: mol_type = other DNA
cagcgccataaacgccaggt

SEQ ID NO: 21 - DNA, 24 bp, synthetic construct
  source 1..24: mol_type = other DNA
tccgcaccgcgcaacgtttccgct

SEQ ID NO: 22 - DNA, 19 bp, synthetic construct
  source 1..19: mol_type = other DNA
ccctgcgtatccagcgaac

SEQ ID NO: 23 - DNA, 22 bp, synthetic construct
  source 1..22: mol_type = other DNA
ttggcttgcttgagcgacaacg

SEQ ID NO: 24 - DNA, 19 bp, synthetic construct
  source 1..19: mol_type = other DNA
ccgccgtccaagctgctga

SEQ ID NO: 25 - DNA, 20 bp, synthetic construct
  source 1..20: mol_type = other DNA
ctcgtccagcgccgcttcgg

SEQ ID NO: 26 - DNA, 18 bp, synthetic construct
  source 1..18: mol_type = other DNA
ccgagaggggacggaaac

SEQ ID NO: 27 - DNA, 18 bp, synthetic construct
  source 1..18: mol_type = other DNA
ccaacagttcatcccggt

SEQ ID NO: 28 - DNA, 16 bp, synthetic construct
  source 1..16: mol_type = other DNA
acgccactgctgaatt

SEQ ID NO: 29 - DNA, 15 bp, synthetic construct
  source 1..15: mol_type = other DNA
ctcgtcgactccttc

SEQ ID NO: 30 - DNA, 15 bp, synthetic construct
  source 1..15: mol_type = other DNA
acttccatcccagtc

SEQ ID NO: 31 - DNA, 15 bp, synthetic construct
  source 1..15: mol_type = other DNA
aagaagtccgcgccg

SEQ ID NO: 32 - DNA, 16 bp, synthetic construct
  source 1..16: mol_type = other DNA
catcacgtcgtggcaa

SEQ ID NO: 33 - DNA, 17 bp, synthetic construct
  source 1..17: mol_type = other DNA
ggtagtccgccgcttcg

SEQ ID NO: 34 - DNA, 17 bp, synthetic construct
  source 1..17: mol_type = other DNA
gcagtcgcccgaacgta

SEQ ID NO: 35 - DNA, 17 bp, synthetic construct
  source 1..17: mol_type = other DNA
tcgccgggtgctctatg

SEQ ID NO: 36 - DNA, 15 bp, synthetic construct
  source 1..15: mol_type = other DNA
atgcgcaccaggctg

SEQ ID NO: 37 - DNA, 17 bp, synthetic construct
  source 1..17: mol_type = other DNA
tttgtgttgtcggtggc

SEQ ID NO: 38 - DNA, 16 bp, synthetic construct
  source 1..16: mol_type = other DNA
taaagtcgaccggcgt

SEQ ID NO: 39 - DNA, 16 bp, synthetic construct
  source 1..16: mol_type = other DNA
tgattccggcaagctg

SEQ ID NO: 40 - DNA, 16 bp, synthetic construct
  source 1..16: mol_type = other DNA
tgccgaaccagcggaa

SEQ ID NO: 41 - DNA, 18 bp, synthetic construct
  source 1..18: mol_type = other DNA
acgccggctacatgtcca

SEQ ID NO: 42 - DNA, 20 bp, synthetic construct
  source 1..20: mol_type = other DNA
cagactggcgtcgctgacat

SEQ ID NO: 43 - DNA, 17 bp, synthetic construct
  source 1..17: mol_type = other DNA
agtctgtggatgcgcct

SEQ ID NO: 44 - DNA, 17 bp, synthetic construct
  source 1..17: mol_type = other DNA
agccgagcgcgatgatg

SEQ ID NO: 45 - DNA, 20 bp, synthetic construct
  source 1..20: mol_type = other DNA
catcctgaccgtggtgttcg

SEQ ID NO: 46 - DNA, 20 bp, synthetic construct
  source 1..20: mol_type = other DNA
acggtgggcaggatgaggta

SEQ ID NO: 47 - DNA, 18 bp, synthetic construct
  source 1..18: mol_type = other DNA
aatcgcctcgtcgccttc

SEQ ID NO: 48 - DNA, 18 bp, synthetic construct
  source 1..18: mol_type = other DNA
gctggaggtgctgatcaa

SEQ ID NO: 49 - DNA, 20 bp, synthetic construct
  source 1..20: mol_type = other DNA
cgtgcaacagttcgtcgagt

SEQ ID NO: 50 - DNA, 19 bp, synthetic construct
  source 1..19: mol_type = other DNA
cgctgatggcattaccgca

SEQ ID NO: 51 - DNA, 17 bp, synthetic construct
  source 1..17: mol_type = other DNA
tcatggccaacgaagtc

SEQ ID NO: 52 - DNA, 18 bp, synthetic construct
  source 1..18: mol_type = other DNA
cggaatactgctcactga

SEQ ID NO: 53 - DNA, 16 bp, synthetic construct
  source 1..16: mol_type = other DNA
cgccgtccctccactc

SEQ ID NO: 54 - DNA, 16 bp, synthetic construct
  source 1..16: mol_type = other DNA
gcatgccgttgatacg

SEQ ID NO: 55 - DNA, 18 bp, synthetic construct
  source 1..18: mol_type = other DNA
cctttgatggcgagcatt

SEQ ID NO: 56 - DNA, 17 bp, synthetic construct
  source 1..17: mol_type = other DNA
gaggagtcctgggtgcc

SEQ ID NO: 57 - DNA, 18 bp, synthetic construct
  source 1..18: mol_type = other DNA
cgcccagatctgtcacca

SEQ ID NO: 58 - DNA, 18 bp, synthetic construct
  source 1..18: mol_type = other DNA
ctgaactgcgccgtgatc

SEQ ID NO: 59 - DNA, 18 bp, synthetic construct
  source 1..18: mol_type = other DNA
ggccagtttgctgccaat

SEQ ID NO: 60 - DNA, 18 bp, synthetic construct
  source 1..18: mol_type = other DNA
gtccagatccgggcagac

SEQ ID NO: 61 - DNA, 17 bp, synthetic construct
  source 1..17: mol_type = other DNA
ataccgcgactggagct

SEQ ID NO: 62 - DNA, 16 bp, synthetic construct
  source 1..16: mol_type = other DNA
gtacggctgcagctca

SEQ ID NO: 63 - DNA, 17 bp, synthetic construct
  source 1..17: mol_type = other DNA
gacgtgattgtcgtaga

SEQ ID NO: 64 - DNA, 18 bp, synthetic construct
  source 1..18: mol_type = other DNA
tttctgggtgtgccgttc

SEQ ID NO: 65 - DNA, 17 bp, synthetic construct
  source 1..17: mol_type = other DNA
ggcgctgcgttggtaga

SEQ ID NO: 66 - DNA, 18 bp, synthetic construct
  source 1..18: mol_type = other DNA
gatttgctgcgcaccgat

SEQ ID NO: 67 - DNA, 17 bp, synthetic construct
  source 1..17: mol_type = other DNA
tctggtcgatgtgctca

SEQ ID NO: 68 - DNA, 18 bp, synthetic construct
  source 1..18: mol_type = other DNA
tagcctacgagctgctgt

SEQ ID NO: 69 - DNA, 16 bp, synthetic construct
  source 1..16: mol_type = other DNA
tagtgagcagcgggaa

SEQ ID NO: 70 - DNA, 17 bp, synthetic construct
  source 1..17: mol_type = other DNA
tgacaatcgtgacgcca

SEQ ID NO: 71 - DNA, 19 bp, synthetic construct
  source 1..19: mol_type = other DNA
tcttccagggtgcgaatga

SEQ ID NO: 72 - DNA, 18 bp, synthetic construct
  source 1..18: mol_type = other DNA
cgagattgccagccttaa

SEQ ID NO: 73 - DNA, 16 bp, synthetic construct
  source 1..16: mol_type = other DNA
atcgtggctgaccgca

SEQ ID NO: 74 - DNA, 19 bp, synthetic construct
  source 1..19: mol_type = other DNA
gggtggatccgatctatga

SEQ ID NO: 75 - DNA, 15 bp, synthetic construct
  source 1..15: mol_type = other DNA
cgtccttggcggtgt

SEQ ID NO: 76 - DNA, 17 bp, synthetic construct
  source 1..17: mol_type = other DNA
ctggaagagctcgtatg

SEQ ID NO: 77 - DNA, 17 bp, synthetic construct
  source 1..17: mol_type = other DNA
ctgtaacgctcatcgcc

SEQ ID NO: 78 - DNA, 15 bp, synthetic construct
  source 1..15: mol_type = other DNA
caactgcgcgctgga

SEQ ID NO: 79 - DNA, 17 bp, synthetic construct
  source 1..17: mol_type = other DNA
gaacgtcttgaagccca

SEQ ID NO: 80 - DNA, 17 bp, synthetic construct
  source 1..17: mol_type = other DNA
acctaccgcatccacga

SEQ ID NO: 81 - DNA, 16 bp, synthetic construct
  source 1..16: mol_type = other DNA
aagctggcgttgtcgg

SEQ ID NO: 82 - DNA, 18 bp, synthetic construct
  source 1..18: mol_type = other DNA
atcgaggaagtgatgacc

SEQ ID NO: 83 - DNA, 17 bp, synthetic construct
  source 1..17: mol_type = other DNA
gtaccttcagattgagc

SEQ ID NO: 84 - DNA, 18 bp, synthetic construct
  source 1..18: mol_type = other DNA
cacccacccattacagaa

SEQ ID NO: 85 - DNA, 18 bp, synthetic construct
  source 1..18: mol_type = other DNA
gcatcctcaccgccctta

SEQ ID NO: 86 - DNA, 18 bp, synthetic construct
  source 1..18: mol_type = other DNA
gaagatggtcgcggtggt

SEQ ID NO: 87 - DNA, 17 bp, synthetic construct
  source 1..17: mol_type = other DNA
ccaatgcccggatgctg

SEQ ID NO: 88 - DNA, 17 bp, synthetic construct
  source 1..17: mol_type = other DNA
cagccgcgaaagcgttg

SEQ ID NO: 89 - DNA, 17 bp, synthetic construct
  source 1..17: mol_type = other DNA
ggctgacgtggggctga

SEQ ID NO: 90 - DNA, 17 bp, synthetic construct
  source 1..17: mol_type = other DNA
cagggcgtcggagacga

SEQ ID NO: 91 - DNA, 16 bp, synthetic construct
  source 1..16: mol_type = other DNA
accggtgcgttgatca

SEQ ID NO: 92 - DNA, 16 bp, synthetic construct
  source 1..16: mol_type = other DNA
ttctgcgggtaagggt

SEQ ID NO: 93 - DNA, 15 bp, synthetic construct
  source 1..15: mol_type = other DNA
gtgactgcaggtgtg

SEQ ID NO: 94 - DNA, 17 bp, synthetic construct
  source 1..17: mol_type = other DNA
agcatctactcgaccaa

SEQ ID NO: 95 - DNA, 17 bp, synthetic construct
  source 1..17: mol_type = other DNA
agcagggacgcgatctc

SEQ ID NO: 96 - DNA, 17 bp, synthetic construct
  source 1..17: mol_type = other DNA
aaccgagcgcatcacca

SEQ ID NO: 97 - DNA, 17 bp, synthetic construct
  source 1..17: mol_type = other DNA
acgggaccgagcgtgtg

SEQ ID NO: 98 - DNA, 17 bp, synthetic construct
  source 1..17: mol_type = other DNA
gcgtttgcggtcgatgc

SEQ ID NO: 99 - DNA, 17 bp, synthetic construct
  source 1..17: mol_type = other DNA
gggcccaacatcggtct

SEQ ID NO: 100 - DNA, 17 bp, synthetic construct
  source 1..17: mol_type = other DNA
ttgcggtacggcgtttc

SEQ ID NO: 101 - DNA, 17 bp, synthetic construct
  source 1..17: mol_type = other DNA
cgggcaacaagctcgac

SEQ ID NO: 102 - DNA, 17 bp, synthetic construct
  source 1..17: mol_type = other DNA
ccttggccatcgaagca

SEQ ID NO: 103 - DNA, 17 bp, synthetic construct
  source 1..17: mol_type = other DNA
ggtcagggcgccagtca

SEQ ID NO: 104 - DNA, 18 bp, synthetic construct
  source 1..18: mol_type = other DNA
ccaggaaccgcacccttg

SEQ ID NO: 105 - DNA, 20 bp, synthetic construct
  source 1..20: mol_type = other DNA
agcactcgatggtgctggtg

SEQ ID NO: 106 - DNA, 20 bp, synthetic construct
  source 1..20: mol_type = other DNA
tgcctgtttgcggttcttga

SEQ ID NO: 107 - DNA, 16 bp, synthetic construct
  source 1..16: mol_type = other DNA
agaagggttgagtgcg

SEQ ID NO: 108 - DNA, 15 bp, synthetic construct
  source 1..15: mol_type = other DNA
gactgtggccggctt

SEQ ID NO: 109 - DNA, 18 bp, synthetic construct
  source 1..18: mol_type = other DNA
gacaccaccgcgctgacc

SEQ ID NO: 110 - DNA, 19 bp, synthetic construct
  source 1..19: mol_type = other DNA
cggtccagcagtacttcgg

SEQ ID NO: 111 - DNA, 18 bp, synthetic construct
  source 1..18: mol_type = other DNA
cggtgggttcaccgaagt

SEQ ID NO: 112 - DNA, 18 bp, synthetic construct
  source 1..18: mol_type = other DNA
caccacccgaggatcgtt

SEQ ID NO: 113 - DNA, 18 bp, synthetic construct
  source 1..18: mol_type = other DNA
ggccgacctgtcgttcat

SEQ ID NO: 114 - DNA, 18 bp, synthetic construct
  source 1..18: mol_type = other DNA
caaactgcggcttcacca

SEQ ID NO: 115 - DNA, 18 bp, synthetic construct
  source 1..18: mol_type = other DNA
ggtccatgacccgcagtt

SEQ ID NO: 116 - DNA, 18 bp, synthetic construct
  source 1..18: mol_type = other DNA
caccgcatcctccaatcc

SEQ ID NO: 117 - DNA, 22 bp, synthetic construct
  source 1..22: mol_type = other DNA
ggaaatcgcagccacgttacgc

SEQ ID NO: 118 - DNA, 22 bp, synthetic construct
  source 1..22: mol_type = other DNA
ccggtaaccaggactgaacggg

SEQ ID NO: 119 - DNA, 18 bp, synthetic construct
  source 1..18: mol_type = other DNA
aacgtgaccgcgaatgtg

SEQ ID NO: 120 - DNA, 18 bp, synthetic construct
  source 1..18: mol_type = other DNA
gatgaccgcaccggagat

SEQ ID NO: 121 - DNA, 19 bp, synthetic construct
  source 1..19: mol_type = other DNA
ctggatgtaccgccgcaac

SEQ ID NO: 122 - DNA, 19 bp, synthetic construct
  source 1..19: mol_type = other DNA
ccgtcgcgcaggaagtaga

SEQ ID NO: 123 - DNA, 17 bp, synthetic construct
  source 1..17: mol_type = other DNA
cacggatccgcgcaagt

SEQ ID NO: 124 - DNA, 17 bp, synthetic construct
  source 1..17: mol_type = other DNA
tcgcgaccgctttttgc

SEQ ID NO: 125 - DNA, 17 bp, synthetic construct
  source 1..17: mol_type = other DNA
gcggtcgcgattcgatg

SEQ ID NO: 126 - DNA, 17 bp, synthetic construct
  source 1..17: mol_type = other DNA
gcgtcggccatcagcac

SEQ ID NO: 127 - DNA, 17 bp, synthetic construct
  source 1..17: mol_type = other DNA
gcgggccgaagtgcttt

SEQ ID NO: 128 - DNA, 17 bp, synthetic construct
  source 1..17: mol_type = other DNA
ggcgcatgcggaagatg

SEQ ID NO: 129 - DNA, 18 bp, synthetic construct
  source 1..18: mol_type = other DNA
caggctcaggaacatctt

SEQ ID NO: 130 - DNA, 16 bp, synthetic construct
  source 1..16: mol_type = other DNA
aagcacgtcacgatgc

SEQ ID NO: 131 - DNA, 17 bp, synthetic construct
  source 1..17: mol_type = other DNA
tgatcggcccgacgaaa

SEQ ID NO: 132 - DNA, 19 bp, synthetic construct
  source 1..19: mol_type = other DNA
cgattggtcgaccgcggaa

SEQ ID NO: 133 - DNA, 17 bp, synthetic construct
  source 1..17: mol_type = other DNA
tacatggccgcggtgct

SEQ ID NO: 134 - DNA, 17 bp, synthetic construct
  source 1..17: mol_type = other DNA
atccatgggcggcacct

SEQ ID NO: 135 - DNA, 19 bp, synthetic construct
  source 1..19: mol_type = other DNA
ttccaggatggcgtagctc

SEQ ID NO: 136 - DNA, 18 bp, synthetic construct
  source 1..18: mol_type = other DNA
ttgacggcctcgacatta

SEQ ID NO: 137 - DNA, 17 bp, synthetic construct
  source 1..17: mol_type = other DNA
aacatccccggccagtc

SEQ ID NO: 138 - DNA, 17 bp, synthetic construct
  source 1..17: mol_type = other DNA
cgcatcgcgtgatcctt

SEQ ID NO: 139 - DNA, 17 bp, synthetic construct
  source 1..17: mol_type = other DNA
cttgggcagctcgtcca

SEQ ID NO: 140 - DNA, 17 bp, synthetic construct
  source 1..17: mol_type = other DNA
ttgacaccgtggtcgtc

SEQ ID NO: 141 - DNA, 18 bp, synthetic construct
  source 1..18: mol_type = other DNA
ttccgggataacggaaca

SEQ ID NO: 142 - DNA, 18 bp, synthetic construct
  source 1..18: mol_type = other DNA
ctcgacgttgtcatcgtg

SEQ ID NO: 143 - DNA, 17 bp, synthetic construct
  source 1..17: mol_type = other DNA
atgccggtcccatagcc

SEQ ID NO: 144 - DNA, 17 bp, synthetic construct
  source 1..17: mol_type = other DNA
cggcgtctgcgatcttc

SEQ ID NO: 145 - DNA, 17 bp, synthetic construct
  source 1..17: mol_type = other DNA
cgtggccatgaggtgct

SEQ ID NO: 146 - DNA, 17 bp, synthetic construct
  source 1..17: mol_type = other DNA
gcctgccgccttgaaat

SEQ ID NO: 147 - DNA, 19 bp, synthetic construct
  source 1..19: mol_type = other DNA
cgggtcgctgaccacgccg

SEQ ID NO: 148 - DNA, 20 bp, synthetic construct
  source 1..20: mol_type = other DNA
tcccagctgcttcgtcgact

SEQ ID NO: 149 - DNA, 21 bp, synthetic construct
  source 1..21: mol_type = other DNA
acgaaggtccgggttctctcg

SEQ ID NO: 150 - DNA, 20 bp, synthetic construct
  source 1..20: mol_type = other DNA
gacaacgctcgcaccctacg

SEQ ID NO: 151 - DNA, 20 bp, synthetic construct
  source 1..20: mol_type = other DNA
gcgtggggagcgaacaggat

SEQ ID NO: 152 - DNA, 20 bp, synthetic construct
  source 1..20: mol_type = other DNA
cttgcggccgtactccccag

SEQ ID NO: 153 - DNA, 20 bp, synthetic construct
  source 1..20: mol_type = other DNA
gccttgtacacaccgcccgt

SEQ ID NO: 154 - DNA, 20 bp, synthetic construct
  source 1..20: mol_type = other DNA
tgatccagccgcaccttccg

SEQ ID NO: 155 - DNA, 20 bp, synthetic construct
  source 1..20: mol_type = other DNA
cgcaagcttcggaggcagac

SEQ ID NO: 156 - DNA, 21 bp, synthetic construct
  source 1..21: mol_type = other DNA
gccgtcggtgaggtaatgcac

SEQ ID NO: 157 - DNA, 20 bp, synthetic construct
  source 1..20: mol_type = other DNA
caacccgaatcagcgcacgt

SEQ ID NO: 158 - DNA, 20 bp, synthetic construct
  source 1..20: mol_type = other DNA
gggacctaccagggcaagga

SEQ ID NO: 159 - DNA, 19 bp, synthetic construct
  source 1..19: mol_type = other DNA
aagaccaggtccacgcggc

SEQ ID NO: 160 - DNA, 19 bp, synthetic construct
  source 1..19: mol_type = other DNA
ctgggcgtgttcaccgagg

SEQ ID NO: 161 - DNA, 19 bp, synthetic construct
  source 1..19: mol_type = other DNA
gagcagcatgtactcggcc

SEQ ID NO: 162 - DNA, 20 bp, synthetic construct
  source 1..20: mol_type = other DNA
gctggccacaacatcacggt

SEQ ID NO: 163 - DNA, 20 bp, synthetic construct
  source 1..20: mol_type = other DNA
ggcgggtcgattgttgggct

SEQ ID NO: 164 - DNA, 23 bp, synthetic construct
  source 1..23: mol_type = other DNA
cgagccgctcaatgaacccaaat

SEQ ID NO: 165 - DNA, 21 bp, synthetic construct
  source 1..21: mol_type = other DNA
tcgccgcgatcaaggagttct

SEQ ID NO: 166 - DNA, 20 bp, synthetic construct
  source 1..20: mol_type = other DNA
ctcacgtgacagaccgccgg

SEQ ID NO: 167 - DNA, 20 bp, synthetic construct
  source 1..20: mol_type = other DNA
tgccaaccatccagcagctg

SEQ ID NO: 168 - DNA, 20 bp, synthetic construct
  source 1..20: mol_type = other DNA
accttccgaagcgccgagtt

SEQ ID NO: 169 - DNA, 22 bp, synthetic construct
  source 1..22: mol_type = other DNA
accatagactcggcgaaattgc

SEQ ID NO: 170 - DNA, 22 bp, synthetic construct
  source 1..22: mol_type = other DNA
tggcgtcgaggtttcacagtct

SEQ ID NO: 171 - DNA, 22 bp, synthetic construct
  source 1..22: mol_type = other DNA
cctaaaccggcgctaaaccgtc

SEQ ID NO: 172 - DNA, 23 bp, synthetic construct
  source 1..23: mol_type = other DNA
tgtcgaagagcggcccttcatgg

SEQ ID NO: 173 - DNA, 21 bp, synthetic construct
  source 1..21: mol_type = other DNA
tcgccgcgatcaaggagttct

SEQ ID NO: 174 - DNA, 20 bp, synthetic construct
  source 1..20: mol_type = other DNA
ctcacgtgacagaccgccgg

SEQ ID NO: 175 - DNA, 20 bp, synthetic construct
  source 1..20: mol_type = other DNA
gctcagggcttcttgtcctt

SEQ ID NO: 176 - DNA, 20 bp, synthetic construct
  source 1..20: mol_type = other DNA
tcgatggggtacttcagggt